European Patent Specification EP 4 060 338 B1, published July 17, 2024. Title: KIT AND METHOD FOR MIXED DETECTION OF PCT AND PRESEPSIN, AND USE THEREOF. Applicant: SHENZHEN MINDRAY BIO-MEDICAL ELECTRONICS CO., LTD. The sequence listing filed with the application follows.

SEQUENCE LISTING (43 sequences)

SEQ ID NO: 1 - protein, 5 aa, Artificial sequence
SVAML

SEQ ID NO: 2 - protein, 5 aa, Artificial sequence
SVEML

SEQ ID NO: 3 - protein, 5 aa, Artificial sequence
SFAML

SEQ ID NO: 4 - protein, 5 aa, Artificial sequence
SFAMA

SEQ ID NO: 5 - protein, 5 aa, Artificial sequence
SVKML

SEQ ID NO: 6 - protein, 5 aa, Artificial sequence
SFKMA

SEQ ID NO: 7 - protein, 17 aa, Artificial sequence
YISYMGSTIYYADAKLG

SEQ ID NO: 8 - protein, 17 aa, Artificial sequence
YISSKSSSNLAADAKLG

SEQ ID NO: 9 - protein, 17 aa, Artificial sequence
YISSGSSTIYYADTVKG

SEQ ID NO: 10 - protein, 17 aa, Artificial sequence
YISSGSSTIYYADMTKG

SEQ ID NO: 11 - protein, 17 aa, Artificial sequence
YITYSGSGAYYADYGNT

SEQ ID NO: 12 - protein, 34 aa, Artificial sequence
YISYMGSTIYYADTVKGYISYMGSTIYYADTVKG

SEQ ID NO: 13 - protein, 17 aa, Artificial sequence
YISSKSSTIYYADTVKG

SEQ ID NO: 14 - protein, 5 aa, Artificial sequence
AGFAY

SEQ ID NO: 15 - protein, 5 aa, Artificial sequence
QQFAY

SEQ ID NO: 16 - protein, 5 aa, Artificial sequence
QGFAY

SEQ ID NO: 17 - protein, 5 aa, Artificial sequence
QGFAM

SEQ ID NO: 18 - protein, 5 aa, Artificial sequence
QQVAY

SEQ ID NO: 19 - protein, 5 aa, Artificial sequence
AGFAM

SEQ ID NO: 20 - protein, 5 aa, Artificial sequence
AGFAY

SEQ ID NO: 21 - protein, 16 aa, Artificial sequence
KSSQSLLYSNGKTYLN

SEQ ID NO: 22 - protein, 16 aa, Artificial sequence
KYYASAAKLYRNIKLN

SEQ ID NO: 23 - protein, 16 aa, Artificial sequence
KYYASLLATYRNIKLN

SEQ ID NO: 24 - protein, 16 aa, Artificial sequence
KYYASLLATTWAKGNN

SEQ ID NO: 25 - protein, 16 aa, Artificial sequence
KSSQSLLYSTWAKGNN

SEQ ID NO: 26 - protein, 16 aa, Artificial sequence
KSSQSLLYSYRNIKLN

SEQ ID NO: 27 - protein, 7 aa, Artificial sequence
LVQSLDS

SEQ ID NO: 28 - protein, 7 aa, Artificial sequence
LVSKLTA

SEQ ID NO: 29 - protein, 7 aa, Artificial sequence
LVSKLDS

SEQ ID NO: 30 - protein, 7 aa, Artificial sequence
LVQSDSK

SEQ ID NO: 31 - protein, 7 aa, Artificial sequence
LQTSDSK

SEQ ID NO: 32 - protein, 7 aa, Artificial sequence
LVSKLAS

SEQ ID NO: 33 - protein, 9 aa, Artificial sequence
VQGTHNYGH

SEQ ID NO: 34 - protein, 9 aa, Artificial sequence
VGGTHFPRT

SEQ ID NO: 35 - protein, 9 aa, Artificial sequence
VGTAIFPRT

SEQ ID NO: 36 - protein, 9 aa, Artificial sequence
VGGTHFITA

SEQ ID NO: 37 - protein, 9 aa, Artificial sequence
VSGTHFPRT

SEQ ID NO: 38 - protein, 9 aa, Artificial sequence
VQGTHFPRT

SEQ ID NO: 39 - protein, 9 aa, Artificial sequence
VQTAIFPRT

SEQ ID NO: 40 - protein, 9 aa, Artificial sequence
VQGTHYGHV

SEQ ID NO: 41 - protein, 9 aa, Artificial sequence
VQGNTFITA

SEQ ID NO: 42 - protein, 12 aa, Artificial sequence
PCELDDEDFRCV

SEQ ID NO: 43 - protein, 64 aa, Artificial sequence
TTPEPCELDDEDFRCVCNFSEPQPDYSEAFQCVSAVEVEIHAGGLNLEPFLKRVDADADPRQYA